European Patent Application EP 4 335 928 A2, published March 13, 2024. Title: QUALITY CONTROL TEMPLATES FOR ENSURING VALIDITY OF SEQUENCING-BASED ASSAYS. Applicant: BILLIONTOONE, INC. The sequence listing filed with the application follows.

SEQUENCE LISTING (61 sequences)

SEQ ID NO: 1 - DNA, 39 bp, synthetic construct
  misc_feature 1..39: note = HBB
  source 1..39: mol_type = other DNA
ggagaagtctgccgttactgccctgtggggcaaggtgaa

SEQ ID NO: 2 - DNA, 39 bp, synthetic construct
  misc_feature 1..39: note = QCT; N may be A, C, T or G
  source 1..39: mol_type = other DNA
ggagaagtnnnnngttactagtctgtnnnnnaaggtgaa

SEQ ID NO: 3 - DNA, 10 bp, synthetic construct
  misc_feature 1..10: note = EMI cluster
  source 1..10: mol_type = other DNA
cattaccgct

SEQ ID NO: 4 - DNA, 10 bp, synthetic construct
  misc_feature 1..10: note = EMI cluster
  source 1..10: mol_type = other DNA
agatccgatt

SEQ ID NO: 5 - DNA, 10 bp, synthetic construct
  misc_feature 1..10: note = EMI cluster
  source 1..10: mol_type = other DNA
ggatcatcgg

SEQ ID NO: 6 - DNA, 10 bp, synthetic construct
  misc_feature 1..10: note = EMI cluster
  source 1..10: mol_type = other DNA
ttacgcgtaa

SEQ ID NO: 7 - DNA, 10 bp, synthetic construct
  misc_feature 1..10: note = EMI cluster
  source 1..10: mol_type = other DNA
tgagttatgg

SEQ ID NO: 8 - DNA, 10 bp, synthetic construct
  misc_feature 1..10: note = EMI cluster
  source 1..10: mol_type = other DNA
taaataatgt

SEQ ID NO: 9 - DNA, 10 bp, synthetic construct
  misc_feature 1..10: note = EMI cluster
  source 1..10: mol_type = other DNA
gtccaactga

SEQ ID NO: 10 - DNA, 10 bp, synthetic construct
  misc_feature 1..10: note = EMI cluster
  source 1..10: mol_type = other DNA
agagtcttat

SEQ ID NO: 11 - DNA, 10 bp, synthetic construct
  misc_feature 1..10: note = EMI cluster
  source 1..10: mol_type = other DNA
tacactcctt

SEQ ID NO: 12 - DNA, 10 bp, synthetic construct
  misc_feature 1..10: note = >Sequence12
  source 1..10: mol_type = other DNA
tgtcatctta

SEQ ID NO: 13 - DNA, 10 bp, synthetic construct
  misc_feature 1..10: note = EMI cluster
  source 1..10: mol_type = other DNA
gtattgcgat

SEQ ID NO: 14 - DNA, 10 bp, synthetic construct
  misc_feature 1..10: note = EMI cluster
  source 1..10: mol_type = other DNA
aatgattaat

SEQ ID NO: 15 - DNA, 10 bp, synthetic construct
  misc_feature 1..10: note = EMI cluster
  source 1..10: mol_type = other DNA
tatatggtca

SEQ ID NO: 16 - DNA, 10 bp, synthetic construct
  misc_feature 1..10: note = EMI cluster
  source 1..10: mol_type = other DNA
ggtgctatag

SEQ ID NO: 17 - DNA, 10 bp, synthetic construct
  misc_feature 1..10: note = EMI cluster
  source 1..10: mol_type = other DNA
gtttaactgg

SEQ ID NO: 18 - DNA, 10 bp, synthetic construct
  misc_feature 1..10: note = EMI cluster
  source 1..10: mol_type = other DNA
acgtgatgta

SEQ ID NO: 19 - DNA, 10 bp, synthetic construct
  misc_feature 1..10: note = EMI cluster
  source 1..10: mol_type = other DNA
tttcatcggt

SEQ ID NO: 20 - DNA, 10 bp, synthetic construct
  misc_feature 1..10: note = EMI cluster
  source 1..10: mol_type = other DNA
cctatccgat

SEQ ID NO: 21 - DNA, 10 bp, synthetic construct
  misc_feature 1..10: note = EMI cluster
  source 1..10: mol_type = other DNA
atagtaacat

SEQ ID NO: 22 - DNA, 10 bp, synthetic construct
  misc_feature 1..10: note = EMI cluster
  source 1..10: mol_type = other DNA
ggactatggt

SEQ ID NO: 23 - DNA, 10 bp, synthetic construct
  misc_feature 1..10: note = EMI cluster
  source 1..10: mol_type = other DNA
aatatagtca

SEQ ID NO: 24 - DNA, 10 bp, synthetic construct
  misc_feature 1..10: note = EMI cluster
  source 1..10: mol_type = other DNA
cttaggtggc

SEQ ID NO: 25 - DNA, 10 bp, synthetic construct
  misc_feature 1..10: note = EMI cluster
  source 1..10: mol_type = other DNA
ctgcctgggc

SEQ ID NO: 26 - DNA, 10 bp, synthetic construct
  misc_feature 1..10: note = EMI cluster
  source 1..10: mol_type = other DNA
ctgccggcgc

SEQ ID NO: 27 - DNA, 10 bp, synthetic construct
  misc_feature 1..10: note = EMI cluster
  source 1..10: mol_type = other DNA
actttcctgc

SEQ ID NO: 28 - DNA, 10 bp, synthetic construct
  misc_feature 1..10: note = EMI cluster
  source 1..10: mol_type = other DNA
tttctcttta

SEQ ID NO: 29 - DNA, 10 bp, synthetic construct
  misc_feature 1..10: note = EMI cluster
  source 1..10: mol_type = other DNA
tttatgggca

SEQ ID NO: 30 - DNA, 10 bp, synthetic construct
  misc_feature 1..10: note = EMI cluster
  source 1..10: mol_type = other DNA
ttgtaggtgc

SEQ ID NO: 31 - DNA, 10 bp, synthetic construct
  misc_feature 1..10: note = EMI cluster
  source 1..10: mol_type = other DNA
ttcggcagaa

SEQ ID NO: 32 - DNA, 10 bp, synthetic construct
  misc_feature 1..10: note = EMI cluster
  source 1..10: mol_type = other DNA
ttcagaatac

SEQ ID NO: 33 - DNA, 10 bp, synthetic construct
  misc_feature 1..10: note = EMI cluster
  source 1..10: mol_type = other DNA
gagctatagc

SEQ ID NO: 34 - DNA, 10 bp, synthetic construct
  misc_feature 1..10: note = EMI cluster
  source 1..10: mol_type = other DNA
cttatcttta

SEQ ID NO: 35 - DNA, 10 bp, synthetic construct
  misc_feature 1..10: note = EMI cluster
  source 1..10: mol_type = other DNA
agataccgtt

SEQ ID NO: 36 - DNA, 10 bp, synthetic construct
  misc_feature 1..10: note = EMI cluster
  source 1..10: mol_type = other DNA
cagatggtat

SEQ ID NO: 37 - DNA, 10 bp, synthetic construct
  misc_feature 1..10: note = EMI cluster
  source 1..10: mol_type = other DNA
ggagtcctgg

SEQ ID NO: 38 - DNA, 10 bp, synthetic construct
  misc_feature 1..10: note = EMI cluster
  source 1..10: mol_type = other DNA
gcctaaaaga

SEQ ID NO: 39 - DNA, 10 bp, synthetic construct
  misc_feature 1..10: note = EMI cluster
  source 1..10: mol_type = other DNA
ggggtggtgt

SEQ ID NO: 40 - DNA, 10 bp, synthetic construct
  misc_feature 1..10: note = EMI cluster
  source 1..10: mol_type = other DNA
taatcgtcta

SEQ ID NO: 41 - DNA, 10 bp, synthetic construct
  misc_feature 1..10: note = EMI cluster
  source 1..10: mol_type = other DNA
gtacagcgca

SEQ ID NO: 42 - DNA, 10 bp, synthetic construct
  misc_feature 1..10: note = EMI cluster
  source 1..10: mol_type = other DNA
tttgtgttat

SEQ ID NO: 43 - DNA, 10 bp, synthetic construct
  misc_feature 1..10: note = EMI cluster
  source 1..10: mol_type = other DNA
gtttcaactt

SEQ ID NO: 44 - DNA, 10 bp, synthetic construct
  misc_feature 1..10: note = EMI cluster
  source 1..10: mol_type = other DNA
tgttaaagat

SEQ ID NO: 45 - DNA, 10 bp, synthetic construct
  misc_feature 1..10: note = EMI cluster
  source 1..10: mol_type = other DNA
gctccttcat

SEQ ID NO: 46 - DNA, 10 bp, synthetic construct
  misc_feature 1..10: note = EMI cluster
  source 1..10: mol_type = other DNA
gtgcgcggtt

SEQ ID NO: 47 - DNA, 10 bp, synthetic construct
  misc_feature 1..10: note = EMI cluster
  source 1..10: mol_type = other DNA
tctatctaag

SEQ ID NO: 48 - DNA, 10 bp, synthetic construct
  misc_feature 1..10: note = EMI cluster
  source 1..10: mol_type = other DNA
tcctgtaaac

SEQ ID NO: 49 - DNA, 10 bp, synthetic construct
  misc_feature 1..10: note = EMI cluster
  source 1..10: mol_type = other DNA
aatagaatgg

SEQ ID NO: 50 - DNA, 10 bp, synthetic construct
  misc_feature 1..10: note = EMI cluster
  source 1..10: mol_type = other DNA
tcatcgtgcg

SEQ ID NO: 51 - DNA, 10 bp, synthetic construct
  misc_feature 1..10: note = EMI cluster
  source 1..10: mol_type = other DNA
tcacgagtac

SEQ ID NO: 52 - DNA, 10 bp, synthetic construct
  misc_feature 1..10: note = EMI cluster
  source 1..10: mol_type = other DNA
tagacaagcg

SEQ ID NO: 53 - DNA, 10 bp, synthetic construct
  misc_feature 1..10: note = EMI cluster
  source 1..10: mol_type = other DNA
cttgtgttat

SEQ ID NO: 54 - DNA, 10 bp, synthetic construct
  misc_feature 1..10: note = EMI cluster
  source 1..10: mol_type = other DNA
cgtgtcttct

SEQ ID NO: 55 - DNA, 10 bp, synthetic construct
  misc_feature 1..10: note = EMI cluster
  source 1..10: mol_type = other DNA
cgatggatga

SEQ ID NO: 56 - DNA, 10 bp, synthetic construct
  misc_feature 1..10: note = EMI cluster
  source 1..10: mol_type = other DNA
cgaaattgcg

SEQ ID NO: 57 - DNA, 10 bp, synthetic construct
  misc_feature 1..10: note = EMI cluster
  source 1..10: mol_type = other DNA
ttttccagct

SEQ ID NO: 58 - DNA, 10 bp, synthetic construct
  misc_feature 1..10: note = EMI cluster
  source 1..10: mol_type = other DNA
tggatattcg

SEQ ID NO: 59 - DNA, 10 bp, synthetic construct
  misc_feature 1..10: note = EMI cluster
  source 1..10: mol_type = other DNA
tattatttaa

SEQ ID NO: 60 - DNA, 10 bp, synthetic construct
  misc_feature 1..10: note = EMI cluster
  source 1..10: mol_type = other DNA
tatccgacta

SEQ ID NO: 61 - DNA, 10 bp, synthetic construct
  misc_feature 1..10: note = EMI cluster
  source 1..10: mol_type = other DNA
tagtcttgtg